European Patent Specification EP 3 480 209 B1, published November 29, 2023. Title: Expression System. Applicant: BLAIS Normand DEHOTTAY Philippe Marc Helene DEWERCHIN Marianne GOFFIN Philippe MARTIN Denis. The sequence listing filed with the application follows.

SEQUENCE LISTING (45 sequences)

SEQ ID NO: 1 - DNA, 72 bp, Artifical Sequence
  misc_signal (0)...(0): PhtE signal sequence
atgaaatttagtaaaaaatatatagcagctggatcagctgttatcgtatccttgagtctatgtgcctatgca

SEQ ID NO: 2 - protein, 24 aa, Artifical Sequence
  SIGNAL (0)...(0): PhtE signal sequence
MKFSKKYIAAGSAVIVSLSLCAYA

SEQ ID NO: 3 - DNA, 75 bp, Artifical Sequence
  misc_signal (0)...(0): SipA signal sequence
atgaaaatgaataaaaaggtactattgacatcgacaatggcagcttcgctattatcagtcgcaagtgttcaagca

SEQ ID NO: 4 - protein, 25 aa, Artifical Sequence
  SIGNAL (0)...(0): SipA signal sequence
MKMNKKVLLTSTMAASLLSVASVQA

SEQ ID NO: 5 - DNA, 63 bp, Artifical Sequence
  misc_signal (0)...(0): OmpA signal sequence
atgaaaaagacagctatcgcgattgcagtggcactggctggtttcgctaccgtagcgcaggcc

SEQ ID NO: 6 - protein, 21 aa, Artifical Sequence
  SIGNAL (0)...(0): OmpA signal sequence
MKKTAIAIAVALAGFATVAQA

SEQ ID NO: 7 - DNA, 57 bp, Artifical Sequence
  misc_signal (0)...(0): NspA signal sequence
atgaaaaaagcacttgccacactgattgccctcgctctcccggccgccgcactggcg

SEQ ID NO: 8 - protein, 19 aa, Artifical Sequence
  SIGNAL (0)...(0): NspA signal sequence
MKKALATLIALALPAAALA

SEQ ID NO: 9 - DNA, 54 bp, Artifical Sequence
  misc_signal (0)...(0): TorT signal sequence
atgcgcgtactgctatttttacttctttcccttttcatgttgccggcattttcg

SEQ ID NO: 10 - protein, 18 aa, Artifical Sequence
  SIGNAL (0)...(0): TorT signal sequence
MRVLLFLLLSLFMLPAFS

SEQ ID NO: 11 - DNA, 69 bp, Artifical Sequence
  misc_signal (0)...(0): SfmC signal sequence
atgatgactaaaataaagttattgatgctcattatattttatttaatcatttcggccagcgcccatgct

SEQ ID NO: 12 - protein, 23 aa, Artifical Sequence
  SIGNAL (0)...(0): SfmC signal sequence
MMTKIKLLMLIIFYLIISASAHA

SEQ ID NO: 13 - DNA, 75 bp, Artifical Sequence
  misc_signal (0)...(0): FocC signal sequence
atgatgaagcacatgcgtatatgggccgttctggcatcatttttagtctttttttatattccgcagagctatgcc

SEQ ID NO: 14 - protein, 25 aa, Artifical Sequence
  SIGNAL (0)...(0): FocC signal sequence
MMKHMRIWAVLASFLVFFYIPQSYA

SEQ ID NO: 15 - DNA, 54 bp, Artifical Sequence
  misc_signal (0)...(0): CcmH signal sequence
atgaggtttttattgggcgtgctgatgctgatgatctccggctcagcgctggcg

SEQ ID NO: 16 - protein, 18 aa, Artifical Sequence
  SIGNAL (0)...(0): CcmH signal sequence
MRFLLGVLMLMISGSALA

SEQ ID NO: 17 - DNA, 69 bp, Artifical Sequence
  misc_signal (0)...(0): YraI signal sequence
atgtcaaaacgaacattcgcggtgatattaaccttgttgtgtagcttctgtattggccaggcgcttgca

SEQ ID NO: 18 - protein, 23 aa, Artifical Sequence
  SIGNAL (0)...(0): YraI signal sequence
MSKRTFAVILTLLCSFCIGQALA

SEQ ID NO: 19 - DNA, 66 bp, Artifical Sequence
  misc_signal (0)...(0): TolB signal sequence
atgatgaagcaggcattacgagtagcatttggttttctcatactgtgggcatcagttctgcatgct

SEQ ID NO: 20 - protein, 22 aa, Artifical Sequence
  SIGNAL (0)...(0): TolB signal sequence
MMKQALRVAFGFLILWASVLHA

SEQ ID NO: 21 - DNA, 66 bp, Artifical Sequence
  misc_signal (0)...(0): NikA signal sequence
atgctctccacactccgccgcactctatttgcgctgctggcttgtgcgtcttttatcgtccatgcc

SEQ ID NO: 22 - protein, 22 aa, Artifical Sequence
  SIGNAL (0)...(0): NikA signal sequence
MLSTLRRTLFALLACASFIVHA

SEQ ID NO: 23 - DNA, 57 bp, Artifical Sequence
  misc_signal (0)...(0): FlgI signal sequence
atgattaaatttctctctgcattaattcttctactggtcacgacggcggctcaggct

SEQ ID NO: 24 - protein, 19 aa, Artifical Sequence
  SIGNAL (0)...(0): FlgI signal sequence
MIKFLSALILLLVTTAAQA

SEQ ID NO: 25 - DNA, 57 bp, Artifical Sequence
  misc_signal (0)...(0)
atgaaaaagatttggctggcgctggctggtttagttttagcgtttagcgcatcggcg

SEQ ID NO: 26 - protein, 19 aa, Artifical Sequence
  SIGNAL (0)...(0): DsbA signal sequence
MKKIWLALAGLVLAFSASA

SEQ ID NO: 27 - DNA, 39 bp, Artifical Sequence
  primer_bind (0)...(0): Primer
gcgcggcatatgggtgcggatgatgtggtggatagcagc

SEQ ID NO: 28 - DNA, 33 bp, Artifical Sequence
  primer_bind (0)...(0): Primer
gcggagctcgagttattagcttttgatttcgaa

SEQ ID NO: 29 - DNA, 90 bp, Artifical Sequence
  primer_bind (0)...(0): Primer
ggagcgcatatgattaaatttctctctgcattaattcttctactggtcacgacggcggctcaggctggtgcggatgatgtggtggatagc

SEQ ID NO: 30 - DNA, 24 bp, Artifical Sequence
  primer_bind (0)...(0): Primer
cacgccgcatagttcgcacccgca

SEQ ID NO: 31 - DNA, 1605 bp, c.diphtheriae
ggtgcggatgatgtggtggatagcagcaaatcttttgtgatggaaaactttagcagctatcatggcaccaaaccgggctatgtggatagcattcagaaaggcatccagaaaccgaaaagcggcacccagggcaactatgatgatgattggaaagaattttatagcaccgataacaaatatgatgcggcgggttatagcgtggataacgaaaatccgctgtctggcaaagcgggcggtgtggtgaaagtgacctatccgggcctgaccaaagtgctggccctgaaagtggataacgcggaaaccatcaaaaaagaactgggcctgagcctgaccgaaccgctgatggaacaggtgggcaccgaagaatttattaaacgctttggcgatggcgcgagccgtgtggttctgagcctgccgtttgcggaaggcagcagcagcgtggaatatattaacaactgggaacaggcgaaagccctgagcgtggaactggaaattaactttgaaacccgtggcaaacgtggccaggatgcgatgtatgaatacatggcgcaggcgtgcgcgggcaatcgtgtgcgtcgtagcgtgggcagcagcctgagctgcattaacctggattgggacgtcattcgtgataaaaccaaaaccaaaatcgaaagcctgaaagaacatggcccgatcaaaaacaaaatgagcgaaagcccgaacaaaaccgtgagcgaagaaaaagcgaaacagtatctggaagaatttcatcagaccgcgctggaacatccggaactgagcgaactgaaaaccgtgaccggcaccaatccggtgtttgcgggtgcgaactatgcggcgtgggcggtgaatgtggcgcaggtgattgatagcgaaaccgcggataacctggaaaaaaccaccgcggccctgagcattctgccgggcattggcagcgtgatgggcattgcggatggcgcggtgcatcataacaccgaagaaattgtggcgcagagcattgccctgagcagcctgatggtggcgcaggcgattccgctggttggcgaactggtggatattggctttgcggcgtacaactttgtggaaagcatcatcaacctgtttcaggtggtgcataacagctataaccgtccggcgtattctccgggtcataaaacccagccgtttctgcatgatggctatgcggtgagctggaacaccgtggaagatagcattattcgtaccggctttcagggcgaaagcggccatgatattaaaattaccgcggaaaacaccccgctgccgattgcgggtgttctgctgccgaccattccgggcaaactggatgtgaacaaaagcaaaacccatattagcgtgaacggtcgtaaaattcgtatgcgttgccgtgcgattgatggcgatgtgaccttttgccgtccgaaaagcccggtgtatgtgggcaacggcgtgcacgcgaacctgcatgtggcgtttcatcgtagcagcagcgaaaaaatccatagcaacgaaattagcagcgatagcattggcgtgctgggctatcagaaaaccgtggaccataccaaagtgaactctaaactgagcctgttcttcgaaatcaaaagc

SEQ ID NO: 32 - protein, 535 aa, c.diphtheriae
GADDVVDSSKSFVMENFSSYHGTKPGYVDSIQKGIQKPKSGTQGNYDDDWKEFYSTDNKYDAAGYSVDNENPLSGKAGGVVKVTYPGLTKVLALKVDNAETIKKELGLSLTEPLMEQVGTEEFIKRFGDGASRVVLSLPFAEGSSSVEYINNWEQAKALSVELEINFETRGKRGQDAMYEYMAQACAGNRVRRSVGSSLSCINLDWDVIRDKTKTKIESLKEHGPIKNKMSESPNKTVSEEKAKQYLEEFHQTALEHPELSELKTVTGTNPVFAGANYAAWAVNVAQVIDSETADNLEKTTAALSILPGIGSVMGIADGAVHHNTEEIVAQSIALSSLMVAQAIPLVGELVDIGFAAYNFVESIINLFQVVHNSYNRPAYSPGHKTQPFLHDGYAVSWNTVEDSIIRTGFQGESGHDIKITAENTPLPIAGVLLPTIPGKLDVNKSKTHISVNGRKIRMRCRAIDGDVTFCRPKSPVYVGNGVHANLHVAFHRSSSEKIHSNEISSDSIGVLGYQKTVDHTKVNSKLSLFFEIKS

SEQ ID NO: 33 - protein, 54 aa, Artifical Sequence
  PhtE signal sequence and the first 30 amino acids of CRM197
MKFSKKYIAAGSAVIVSLSLCAYAGADDVVDSSKSFVMENFSSYHGTKPGYVDS

SEQ ID NO: 34 - protein, 55 aa, Artifical Sequence
  SipA signal sequence and the first 30 amino acids of CRM197
MKMNKKVLLTSTMAASLLSVASVQAGADDVVDSSKSFVMENFSSYHGTKPGYVDS

SEQ ID NO: 35 - protein, 51 aa, Artifical Sequence
  OmpA signal sequence and the first 30 amino acids of CRM197
MKKTAIAIAVALAGFATVAQAGADDVVDSSKSFVMENFSSYHGTKPGYVDS

SEQ ID NO: 36 - protein, 49 aa, Artifical Sequence
  NspA signal sequence and the first 30 amino acids of CRM197
MKKALATLIALALPAAALAGADDVVDSSKSFVMENFSSYHGTKPGYVDS

SEQ ID NO: 37 - protein, 48 aa, Artifical Sequence
  TorT signal sequence and the first 30 amino acids of CRM197
MRVLLFLLLSLFMLPAFSGADDVVDSSKSFVMENFSSYHGTKPGYVDS

SEQ ID NO: 38 - protein, 53 aa, Artifical Sequence
  SfmC signal sequence and the first 30 amino acids of CRM197
MMTKIKLLMLIIFYLIISASAHAGADDVVDSSKSFVMENFSSYHGTKPGYVDS

SEQ ID NO: 39 - protein, 55 aa, Artifical Sequence
  FocC signal sequence and the first 30 amino acids of CRM197
MMKHMRIWAVLASFLVFFYIPQSYAGADDVVDSSKSFVMENFSSYHGTKPGYVDS

SEQ ID NO: 40 - protein, 48 aa, Artifical Sequence
  CcmH signal sequence and the first 30 amino acids of CRM197
MRFLLGVLMLMISGSALAGADDVVDSSKSFVMENFSSYHGTKPGYVDS

SEQ ID NO: 41 - protein, 53 aa, Artifical Sequence
  YraI signal sequence and the first 30 amino acids of CRM197
MSKRTFAVILTLLCSFCIGQALAGADDVVDSSKSFVMENFSSYHGTKPGYVDS

SEQ ID NO: 42 - protein, 52 aa, Artifical Sequence
  TolB signal sequence and the first 30 amino acids of CRM197
MMKQALRVAFGFLILWASVLHAGADDVVDSSKSFVMENFSSYHGTKPGYVDS

SEQ ID NO: 43 - protein, 52 aa, Artifical Sequence
  NikA signal sequence and the first 30 amino acids of CRM197
MLSTLRRTLFALLACASFIVHAGADDVVDSSKSFVMENFSSYHGTKPGYVDS

SEQ ID NO: 44 - protein, 49 aa, Artifical Sequence
  FlgI signal sequence and the first 30 amino acids of CRM197
MIKFLSALILLLVTTAAQAGADDVVDSSKSFVMENFSSYHGTKPGYVDS

SEQ ID NO: 45 - protein, 49 aa, Artifical Sequence
  DsbA signal sequence and the first 30 amino acids of CRM197
MKKIWLALAGLVLAFSASAGADDVVDSSKSFVMENFSSYHGTKPGYVDS